European Patent Specification EP 3 444 279 B1, published July 26, 2023. Title: ANTIBODY HAVING IMPROVED STABILITY AND SPECIFICALLY BINDING TO HER2. Applicant: AbClon Inc. Application EP 17782617.9. The sequence listing filed with the application follows.

SEQUENCE LISTING (22 sequences)

SEQ ID NO: 1 - protein, 5 aa, Artificial Sequence
  CDRH1 of hz1E11 antibody
SYTMS

SEQ ID NO: 2 - protein, 17 aa, Artificial Sequence
  CDRH2 of hz1E11 antibody
YISNGGGSTYYPDTVKG

SEQ ID NO: 3 - protein, 10 aa, Artificial Sequence
  CDRH3 of hz1E11 antibody
HLGGTASFDY

SEQ ID NO: 4 - protein, 11 aa, Artificial Sequence
  CDRL1 of hz1E11 antibody
LASQTIGTWLA

SEQ ID NO: 5 - protein, 6 aa, Artificial Sequence
  CDRL2 of hz1E11 antibody
ATSLAD

SEQ ID NO: 6 - protein, 9 aa, Artificial Sequence
  CDRL3 of hz1E11 antibody
QQLYSTPWT

SEQ ID NO: 7 - protein, 119 aa, Artificial Sequence
  Amino acid sequence of hz1E11 heavy chain variable region
EVQLVESGGGLVQPGGSLRLSCAASGFTFSSYTMSWVRQAPGKGLEWVAYISNGGGSTYYPDTVKGRFTISRDNAKNSLYLQMNSLRAEDTAVYYCARHLGGTASFDYWGQGTLVTVSS

SEQ ID NO: 8 - protein, 107 aa, Artificial Sequence
  Amino acid sequence of hz1E11 light chain variable region
DIQMTQSPSSLSASVGDRVTITCLASQTIGTWLAWYQQKPGKAPKLLIYVATSLADGVPSRFSGSGSGTDFTLTISSLQPEDFATYYCQQLYSTPWTFGQGTKVEIK

SEQ ID NO: 9 - protein, 17 aa, Artificial Sequence
  CDRH2 of hz1E11.10
YISAGGGSTYYPDTVKG

SEQ ID NO: 10 - protein, 17 aa, Artificial Sequence
  CDRH2 of hz1E11.20
YISNAGGSTYYPDTVKG

SEQ ID NO: 11 - protein, 17 aa, Artificial Sequence
  CDRH2 of hz1E11.10/20
YISAAGGSTYYPDTVKG

SEQ ID NO: 12 - protein, 107 aa, Artificial Sequence
  Amino acid sequence of hzlE11.01 light chain variable region
DIQMTQSPSSLSASVGDRVTITCLASQTIGTWLAWYQQKPGKAPKLLIYVATSLAAGVPSRFSGSGSGTDFTLTISSLQPEDFATYYCQQLYSTPWTFGQGTKVEIK

SEQ ID NO: 13 - protein, 107 aa, Artificial Sequence
  Amino acid sequence of hzlE11.02 light chain variable region
DIQMTQSPSSLSASVGDRVTITCLASQTIGTWLAWYQQKPGKAPKLLIYVATSLADAVPSRFSGSGSGTDFTLTISSLQPEDFATYYCQQLYSTPWTFGQGTKVEIK

SEQ ID NO: 14 - protein, 107 aa, Artificial Sequence
  Amino acid sequence of hzlE11.01/02 light chain variable region
DIQMTQSPSSLSASVGDRVTITCLASQTIGTWLAWYQQKPGKAPKLLIYVATSLAAAVPSRFSGSGSGTDFTLTISSLQPEDFATYYCQQLYSTPWTFGQGTKVEIK

SEQ ID NO: 15 - DNA, 32 bp, Artificial Sequence
  primer F_N52aA
gtagcctacatctccgccgggggcggaagtac

SEQ ID NO: 16 - DNA, 32 bp, Artificial Sequence
  primer R_N52aA
gtacttccgcccccggcggagatgtaggctac

SEQ ID NO: 17 - DNA, 30 bp, Artificial Sequence
  primer F_G53A
ctacatctccaacgccggcggaagtacgta

SEQ ID NO: 18 - DNA, 30 bp, Artificial Sequence
  primer R_G53A
tacgtacttccgccggcgttggagatgtag

SEQ ID NO: 19 - DNA, 33 bp, Artificial Sequence
  primer F_D56A
gcaacgagtctcgctgccggtgtgccttccaga

SEQ ID NO: 20 - DNA, 33 bp, Artificial Sequence
  primer R_D56A
tctggaaggcacaccggcagcgagactcgttgc

SEQ ID NO: 21 - DNA, 32 bp, Artificial Sequence
  primer F_G57A
cgagtctcgctgacgccgtgccttccagattt

SEQ ID NO: 22 - DNA, 32 bp, Artificial Sequence
  primer R_G57A
aaatctggaaggcacggcgtcagcgagactcg